European Patent Specification EP 3 068 216 B1, published April 10, 2024. Title: METHOD OF PRODUCING INFERTILE FISH AND EGG-PRODUCING AQUATIC ANIMALS AND OF  DELIVERING COMPOUNDS INTO EGGS AND EMBRYOS. Applicant: UNIVERSITY OF MARYLAND BALTIMORE COUNTY. Application Not yet assigned. The sequence listing filed with the application follows.

SEQUENCE LISTING (5 sequences)

SEQ ID NO: 1 - DNA, 25 bp, Salmo salar
ctgacttgaacgctcctccattatc

SEQ ID NO: 2 - DNA, 18 bp, Salmo salar
acttgaacgctcctccat

SEQ ID NO: 3 - DNA, 25 bp, Morone saxatilis
ggctctgcttgctctccatcatctc

SEQ ID NO: 4 - DNA, 25 bp, Oreochromi niloticus
ctggctttgcgtgttttccatcgtc

SEQ ID NO: 5 - DNA, 25 bp, Danio rerio
gctgggcatccatgtctccgaccat